European Patent Application EP 4 477 071 A2, published December 18, 2024. Title: Tolerance in plants of Solanum lycopersicum to the tobamovirus Tomato Brown Rugose Fruit virus (TBRFV). Applicant: VILMORIN & CIE. Application EP. The sequence listing filed with the application follows.

SEQUENCE LISTING (18 sequences)

SEQ ID NO: 1 - DNA, 121 bp, Lycopersicon esculentum
  misc_feature 61: note = polymorphism - susceptible = C; tolerant = T
  source 1..121: mol_type = other DNA
gtcggaccaagaaaccatatttggtaacgggttcgagttgctgcctgaaccttttagcccyttgcaatatttgtgaagtgatattcctttgtgttattaataatttttcgttttgagtttt

SEQ ID NO: 2 - DNA, 121 bp, Lycopersicon esculentum
  misc_feature 61: note = polymorphism - susceptible = T; tolerant = C
  source 1..121: mol_type = other DNA
ttcagagagcaacactcctgcaagaccaactcggagtaattcagtaactcgaccttccatytctagctctcagtatagtacttactcaaataaatcaggctctattctaaacacaagctct

SEQ ID NO: 3 - DNA, 101 bp, Lycopersicon esculentum
  misc_feature 51: note = polymorphism - susceptible = A; tolerant = G
  source 1..101: mol_type = other DNA
ttccgaaatgaggacgatccatcagcttcttcagctgagagcccctggtcracataccagaattctgtttttctaaaactgtccaaaatctcctgtaaaga

SEQ ID NO: 4 - DNA, 71 bp, Lycopersicon esculentum
  misc_feature 36: note = polymorphism - susceptible = T; tolerant = C
  source 1..71: mol_type = other DNA
gatttgaatgccttgccacagccagaggatgacgaygagatttttggacaacaattagaagatgaaccaca

SEQ ID NO: 5 - DNA, 121 bp, Lycopersicon esculentum
  misc_feature 61: note = polymorphism - susceptible = A; tolerant = G
  source 1..121: mol_type = other DNA
agagaatgatatcactgccttagtttctcaattaaaagttgtgcaaaaacaaaacacacarctagatgaagaaaacagagcattcgcctcaaagcttcagacaaaagaagttgagaacaac

SEQ ID NO: 6 - DNA, 71 bp, Lycopersicon esculentum
  misc_feature 36: note = polymorphism - susceptible = T; tolerant = G
  source 1..71: mol_type = other DNA
tacaataccttctggcatccctttccgcaaaacgakagatctttagtatcaaaaccgagagcactgtcacc

SEQ ID NO: 7 - DNA, 101 bp, Lycopersicon esculentum
  misc_feature 51: note = polymorphism - susceptible = A; tolerant = T
  source 1..101: mol_type = other DNA
atggcaatagtgaactgcagatacaactgaaattgcagaacacccttaaawatagaatcaatagaaagttgcaacaatatttgaatgatgaagcaacaaag

SEQ ID NO: 8 - DNA, 101 bp, Lycopersicon esculentum
  misc_feature 51: note = polymorphism - susceptible = T; tolerant = C
  source 1..101: mol_type = other DNA
agccattgtgattgtgtctgttgtacattaccaaaattctctagagaaagygatacacatgccagccctatcgatataaagcaacgcaaggtggattctgc

SEQ ID NO: 9 - DNA, 101 bp, Lycopersicon esculentum
  misc_feature 51: note = polymorphism - susceptible = C; tolerant = T
  source 1..101: mol_type = other DNA
aacaccaggtagagagcacagcgaaacaatggcctcaggaagatctacttygcgaagtgcagcaagccactccatacctccaccaggctttgatttcagtg

SEQ ID NO: 10 - DNA, 101 bp, Lycopersicon esculentum
  misc_feature 51: note = polymorphism - susceptible = A; tolerant = G
  source 1..101: mol_type = other DNA
tcaactgcaactttaacagctgattcaacttcttcttctttcgaaacatcrcattgaatgtaacgacctccaatagattcagctaaacttgtacctacttc

SEQ ID NO: 11 - DNA, 101 bp, Lycopersicon esculentum
  misc_feature 51: note = polymorphism - susceptible = C; tolerant = A
  source 1..101: mol_type = other DNA
gaggagctatcaacttcatagtcagattcagaaaatgattcagatgaggamgtggctgattcttcttgttttcttttcttccttctgctcgaactctctcc

SEQ ID NO: 12 - DNA, 101 bp, Lycopersicon esculentum
  misc_feature 51: note = polymorphism - susceptible = G; tolerant = A
  source 1..101: mol_type = other DNA
cagaaataatagaaaatcagaaagaaaaatcagctttctaaatggaaaagrcgatggcactatgtttgaagttttaagcaacttttctgaagtcccaaaag

SEQ ID NO: 13 - DNA, 160 bp, Lycopersicon esculentum
  misc_feature 59: note = polymorphism - susceptible = A; tolerant = G
  source 1..160: mol_type = other DNA
ctcctattgaacatcctgaaaacttgtgtctacatcatgagaagatgcaggccaattcrctcagtacatggaatgcacgagcatgttaggggaattctaacgcaaagcataagcttgatacttgaataaaagatgaaacatacttacttcttctcaaact

SEQ ID NO: 14 - DNA, 101 bp, Lycopersicon esculentum
  misc_feature 51: note = polymorphism - susceptible = A; tolerant = G
  source 1..101: mol_type = other DNA
ctcttggtgacaaaccactggctcaatttcttcgcgaagctaaagctatcrctgatgagcttgtcacggcaggcacacgtgtctcctgatgaattcaatgc

SEQ ID NO: 15 - DNA, 101 bp, Lycopersicon esculentum
  misc_feature 51: note = polymorphism - susceptible = T; tolerant = G
  source 1..101: mol_type = other DNA
cattactgttgagatatctcatcggcaacccctggagcttgcccacccgcktgtcctccaggatctgatttcagaaaggatgaatagtaactgtgtttcag

SEQ ID NO: 16 - DNA, 121 bp, Lycopersicon esculentum
  misc_feature 61: note = polymorphism - susceptible = G; tolerant = A
  source 1..121: mol_type = other DNA
caagaacccaacgacttcttcttctttgcttattgaaaaacttggttttgaaatgaaaggratcgagaaattggatactcagtggttctctactactaaaccttctcctgattttaagaaa

SEQ ID NO: 17 - DNA, 101 bp, Lycopersicon esculentum
  misc_feature 51: note = polymorphism - susceptible = T; tolerant = C
  source 1..101: mol_type = other DNA
tgatcgacaattcttgttgttgttgaaactctgcaagtgagagagggatgyatatagagaaaggatattggtaaaggacaattctagaagggtctagggaa

SEQ ID NO: 18 - DNA, 101 bp, Lycopersicon esculentum
  misc_feature 51: note = polymorphism - susceptible = C; tolerant = T
  source 1..101: mol_type = other DNA
gcaccagttatagtaatgtcctgcttctttcctgtacccttatcagtagcygtgacagaaagaataccgttggtgtcaatgtcgaacttcacttcaatctg